European Patent Specification EP 3 600 389 B1, published May 10, 2023. Title: METHODS AND COMPOSITIONS FOR STIMULATING IMMUNE RESPONSE. Applicant: BioNTech RNA Pharmaceuticals GmbH. The sequence listing filed with the application follows.

SEQUENCE LISTING (12 sequences)

SEQ ID NO: 1 - RNA, 17 nt, Artificial Sequence
  Sequence of immunostimulatory RNA molecule
aacuucuggagggguga

SEQ ID NO: 2 - RNA, 21 nt, Artificial Sequence
  Sequence of immunostimulatory RNA molecule
aacuucuggaggggugagaau

SEQ ID NO: 3 - RNA, 6 nt, Artificial Sequence
  Sequence of immunostimulatory RNA molecule
uugcuu

SEQ ID NO: 4 - RNA, 11 nt, Artificial Sequence
  Sequence of immunostimulatory RNA molecule
aagaauugcuu

SEQ ID NO: 5 - RNA, 38 nt, Artificial Sequence
  Sequence of immunostimulatory RNA molecule
gggcgaacuaguaacuucuggaggggugagaaucucga

SEQ ID NO: 6 - RNA, 23 nt, Artificial Sequence
  Sequence of immunostimulatory RNA molecule
aacuucuggaggggugauugcuu

SEQ ID NO: 7 - RNA, 40 nt, Artificial Sequence
  Sequence of immunostimulatory RNA molecule
gggcgaacuaguaacuucuggaggggugauugcuucucga

SEQ ID NO: 8 - RNA, 43 nt, Artificial Sequence
  Sequence of immunostimulatory RNA molecule
aacuucuggaggggugagaauggacgaaaaacaagaauugcuu

SEQ ID NO: 9 - RNA, 60 nt, Artificial Sequence
  Sequence of immunostimulatory RNA molecule
gggcgaacuaguaacuucuggaggggugagaauggacgaaaaacaagaauugcuucucga

SEQ ID NO: 10 - RNA, 32 nt, Artificial Sequence
  Sequence of immunostimulatory RNA molecule
aacuucuggaggggugagaauaagaauugcuu

SEQ ID NO: 11 - RNA, 49 nt, Artificial Sequence
  Sequence of immunostimulatory RNA molecule
gggcgaacuaguaacuucuggaggggugagaauaagaauugcuucucga

SEQ ID NO: 12 - RNA, 1565 nt, Influenza A virus
agcaaaagcaggguagauaaucacucacugagugacaucaaaaucauggcgucucaaggcaccaaacgaucuuacgaacagauggagacugauggagaacgccagaaugccacugaaaucagagcauccgucggaaaaaugauugguggaauuggacgauucuacauccaaaugugcaccgaacucaaacucagugauuaugagggacgguugauccaaaacagcuuaacaauagagagaauggugcucucugcuuuugacgaaaggagaaauaaauaccuugaagaacaucccagugcggggaaagauccuaagaaaacuggaggaccuauauacaggagaguaaacggaaaguggaugagagaacucauccuuuaugacaaagaagaaauaaggcgaaucuggcgccaagcuaauaauggugacgaugcaacggcuggucugacucacaugaugaucuggcauuccaauuugaaugaugcaacuuaucagaggacaagagcucuuguucgcaccggaauggaucccaggaugugcucucugaugcaagguucaacucucccuaggaggucuggagccgcaggugcugcagucaaaggaguuggaacaauggugauggaauuggucagaaugaucaaacgugggaucaaugaucggaacuucuggaggggugagaauggacgaaaaacaagaauugcuuaugaaagaaugugcaacauucucaaagggaaauuucaaacugcugcacaaaaagcaaugauggaucaagugagagagagccggaacccagggaaugcugaguucgaagaucucacuuuucuagcacggucugcacucauauugagagggucgguugcucacaaguccugccugccugccuguguguauggaccugccguagccaguggguacgacuuugaaagggagggauacucucuagucggaauagacccuuucagacugcuucaaaacagccaaguguacagccuaaucagaccaaaugagaauccagcacacaagagucaacugguguggauggcaugccauucugccgcauuugaagaucuaagaguauuaagcuucaucaaagggacgaaggugcucccaagagggaagcuuuccacuagaggaguucaaauugcuuccaaugaaaauauggagacuauggaaucaaguacacuugaacugagaagcagguacugggccauaaggaccagaaguggaggaaacaccaaucaacagagggcaucugcgggccaaaucagcauacaaccuacguucucaguacagagaaaucucccuuuugacagaacaaccguuauggcagcauucagugggaauacagaggggagaacaucugacaugaggaccgaaaucauaaggaugauggaaagugcaagaccagaagaugugucuuuccaggggcggggagucuucgagcucucggacgaaaaggcagcgagcccgaucgugccuuccuuugacaugaguaaugaaggaucuuauuucuucggagacaaugcagaggaauacgauaauuaaagaaaaauacccuuguuucuacu